European Patent Specification EP 3 244 932 B1, published March 5, 2025. Title: RNA Guided Eradication of Herpes Simplex Type I and Other Related Human Herpesviruses. Applicant: TEMPLE UNIVERSITY-OF THE COMMONWEALTH SYSTEM OF HIGHER EDUCATION Roehm, Pamela C Khalili, Kamel Shekarabi, Seyed Masoud Wollebo, Hassen. The sequence listing filed with the application follows.

SEQUENCE LISTING (56 sequences)

SEQ ID NO: 1 - DNA, 30 bp, herpes simplex virus
tctgggtgtttccctgcgaccgagacctgc

SEQ ID NO: 2 - DNA, 31 bp, herpes simplex virus
ggacagcacggacacggaactgttcgagacg

SEQ ID NO: 3 - DNA, 20 bp, herpes simplex virus
gcatcccgtgcatgaaaacc

SEQ ID NO: 4 - DNA, 30 bp, herpes simplex virus
tgtgcaacgccaagctggtgtacctgatag

SEQ ID NO: 5 - DNA, 20 bp, herpes simplex virus
gcgagtacccgccggcctga

SEQ ID NO: 6 - DNA, 20 bp, herpes simplex virus
gcgagccgcggcgccgcggg

SEQ ID NO: 7 - DNA, 20 bp, herpes simplex virus
ttctacgcgcgctatcgcga

SEQ ID NO: 8 - DNA, 20 bp, herpes simplex virus
ggagtgttcctcgtcggacg

SEQ ID NO: 9 - DNA, 33 bp, herpes simplex virus
tctgggtgtttccctgcgaccgagacctgccgg

SEQ ID NO: 10 - DNA, 34 bp, herpes simplex virus
ggacagcacggacacggaactgttcgagacgggg

SEQ ID NO: 11 - DNA, 23 bp, herpes simplex virus
gcatcccgtgcatgaaaacctgg

SEQ ID NO: 12 - DNA, 33 bp, herpes simplex virus
tgtgcaacgccaagctggtgtacctgatagtgg

SEQ ID NO: 13 - DNA, 23 bp, herpes simplex virus
gcgagtacccgccggcctgaggg

SEQ ID NO: 14 - DNA, 23 bp, herpes simplex virus
gcgagccgcggcgccgcgggggg

SEQ ID NO: 15 - DNA, 23 bp, herpes simplex virus
ttctacgcgcgctatcgcgacgg

SEQ ID NO: 16 - DNA, 23 bp, herpes simplex virus
ggagtgttcctcgtcggacgagg

SEQ ID NO: 17 - DNA, 19 bp, Artificial Sequence
  chemically synthesized
gatgtctgggtgtttccct

SEQ ID NO: 18 - DNA, 26 bp, Artificial Sequence
  chemically synthesized
cacgatcgggatggtgctgaacgacc

SEQ ID NO: 19 - DNA, 21 bp, Artificial Sequence
  chemically synthesized
tgctgattgacgcgggaaatc

SEQ ID NO: 20 - DNA, 20 bp, Artificial Sequence
  chemically synthesized
cgatctcatccgtgcacacg

SEQ ID NO: 21 - DNA, 24 bp, Artificial Sequence
  chemically synthesized
ccatccacgccctgcggccccagc

SEQ ID NO: 22 - DNA, 20 bp, Artificial Sequence
  chemically synthesized
cacgtctgtgggtgttcaga

SEQ ID NO: 23 - DNA, 20 bp, Artificial Sequence
  chemically synthesized
aaagctcctagggctgttgg

SEQ ID NO: 24 - DNA, 20 bp, Artificial Sequence
  chemically synthesized
ggaaccccctcgctttcttt

SEQ ID NO: 25 - DNA, 20 bp, Artificial Sequence
  chemically synthesized
cgtatgtgtcccatcggcat

SEQ ID NO: 26 - DNA, 20 bp, Artificial Sequence
  chemically synthesized
cactgccttgtgcccataga

SEQ ID NO: 27 - DNA, 20 bp, Artificial Sequence
  chemically synthesized
ttgaagctgcacgtgttgga

SEQ ID NO: 28 - DNA, 20 bp, Artificial Sequence
  chemically synthesized
actgacgggatctgggatca

SEQ ID NO: 29 - DNA, 20 bp, Artificial Sequence
  chemically synthesized
ttcactgggagacgtcaagc

SEQ ID NO: 30 - DNA, 20 bp, Artificial Sequence
  chemically synthesized
gtgaggccccacacatgatt

SEQ ID NO: 31 - DNA, 21 bp, Artificial Sequence
  chemically synthesized
aaggatgagagatggggaagc

SEQ ID NO: 32 - DNA, 38 bp, Artificial Sequence
  chemically synthesized
tatgggcccacgcgtgagggcctatttcccatgattcc

SEQ ID NO: 33 - DNA, 38 bp, Artificial Sequence
  chemically synthesized
tgtggatcctcgaggcgggccatttaccgtaagttatg

SEQ ID NO: 34 - DNA, 23 bp, Artificial Sequence
  chemically synthesized
tccctgcgaccgagacctgccgg

SEQ ID NO: 35 - DNA, 23 bp, Artificial Sequence
  chemically synthesized
acacggaactgttcgagacgggg

SEQ ID NO: 36 - DNA, 23 bp, Artificial Sequence
  chemically synthesized
gcatcccgtgcatgaaaacctgg

SEQ ID NO: 37 - DNA, 46 bp, Artificial Sequence
  chemically synthesized
  misc_feature (1)..(10): n is a, c, g, or t
  misc_feature (12)..(30): n is a, c, g, or t
  misc_feature (33)..(46): n is a, c, g, or t
nnnnnnnnnngnnnnnnnnnnnnnnnnnnnggnnnnnnnnnnnnnn

SEQ ID NO: 38 - DNA, 46 bp, Artificial Sequence
  chemically synthesized
  misc_feature (1)..(10): n is a, c, g, or t
  misc_feature (12)..(30): n is a, c, g, or t
  misc_feature (33)..(46): n is a, c, g, or t
nnnnnnnnnncnnnnnnnnnnnnnnnnnnnccnnnnnnnnnnnnnn

SEQ ID NO: 39 - RNA, 119 nt, Artificial Sequence
  chemically synthesized
  misc_feature (2)..(20): n is a, c, g, or u
gnnnnnnnnnnnnnnnnnnnguuuuagagcuagaaauagcaaguuaaaauaaggcuaguccguuaucaacuugaaaaaguggcaccgacuugaaaaaguggcaccgagcguggcuuuuu

SEQ ID NO: 40 - DNA, 48 bp, herpes simplex virus
cccgccccggatgtctgggtgttccctgcgaccgagactgccggacag

SEQ ID NO: 41 - DNA, 31 bp, herpes simplex virus
ttctgcatcccgtgcatgaaaacctggatgc

SEQ ID NO: 42 - DNA, 51 bp, Artificial Sequence
  chemically synthesized
ccccccgccccggatgtctgggtgttccctgcgaccgagacacctggatgc

SEQ ID NO: 43 - DNA, 52 bp, Artificial Sequence
  chemically synthesized
ccccccgccccggatgtctgggtgttccctgcgaccgagacaacctggatgc

SEQ ID NO: 44 - DNA, 52 bp, Artificial Sequence
  chemically synthesized
ccccccgccccggatgtctgggtgttccctgcgaccgagacgacctggatgc

SEQ ID NO: 45 - DNA, 30 bp, Artificial Sequence
  chemically synthesized
gtttccctgcgaccgagaccacctggatgc

SEQ ID NO: 46 - DNA, 65 bp, Artificial Sequence
  chemically synthesized
atgtctgggtgtttccctgcgaccgagacctgccggacagcagcgactctgaggcggagaccgaa

SEQ ID NO: 47 - DNA, 65 bp, Artificial Sequence
  chemically synthesized
atgtctgggtgtttccctgcgaccgagacctgccggacaagcagcgactcggaggcggagaccga

SEQ ID NO: 48 - DNA, 65 bp, Artificial Sequence
  chemically synthesized
atgtctgggtgtttccctgcgaccgagacctgccggacagcagcgactcggaggcggagacgaag

SEQ ID NO: 49 - DNA, 30 bp, Artificial Sequence
  chemically synthesized
atgtctgggtgtttccctgcgaccgagacc

SEQ ID NO: 50 - DNA, 31 bp, Artificial Sequence
  chemically synthesized
gtttccctgcgaccgagaccaacctggatgc

SEQ ID NO: 51 - DNA, 31 bp, Artificial Sequence
  chemically synthesized
gtttccctgcgaccgagaccgacctggatgc

SEQ ID NO: 52 - DNA, 23 bp, Homo sapiens
cctgcaggtctctttcccatgga

SEQ ID NO: 53 - DNA, 23 bp, Homo sapiens
cccgagcgaccgagaccagccgg

SEQ ID NO: 54 - DNA, 23 bp, Homo sapiens
tcctggccaccgagacctgaagg

SEQ ID NO: 55 - DNA, 23 bp, Homo sapiens
tgccagataccgagacctgcgag

SEQ ID NO: 56 - DNA, 24 bp, Homo sapiens
tccctgcgccaagggacctgccag